European Patent Specification EP 3 707 238 B1, published April 23, 2025. Title: Micro-organism tolerant for inorganic nitrogen compounds. Applicant: Biosolum B.V. The sequence listing filed with the application follows.

SEQUENCE LISTING (94 sequences)

SEQ ID NO: 1 - DNA, 115 bp, Unknown
  newly identified micro-organism
tacgaccatagggtgtggaaaacagggcttcccgtccgctcagccgtacttaagccacacgccggccggttagtagttgggtgggtgaccaccagcgaatcccggctgttgtatg

SEQ ID NO: 2 - DNA, 115 bp, Unknown
  Newly identified micro-organism
atacaacagccgggattcgctggtggtcacccacccaactactaaccggccggcgtgtggcttaagtacggctgagcggacgggaagccctgttttccacaccctatggtcgtat

SEQ ID NO: 3 - DNA, 112 bp, Unknown
  Newly identified micro-organism
acgaccatagggtgtggaaaacagggcttcccgtccgctcagccgtacttaagccacacgccggccggttagtagttgggtgggtgaccaccagcgaatcccggctgttgta

SEQ ID NO: 4 - DNA, 1280 bp, Unknown
  Newly identified micro-organism
tcctcctttcggcgcttgacgagttgttagtaccaaactgaaggaaaattcaccgtgacgatggtgattcacgattactagtaattccttattcatgtagtcgagttacagactacaatccatattatatccatttttggggattagctcaatttcgcaatgtcgcatccctttgttatggcgtatgtggcacgtctgtagcccacagtatttaggccatgatgacttgtcttaatccctattacatacctagataatggtgaaccactttatgtatgtaaataaagtgaggggtttcgttaattataggtaattaccaaatctcacgacatcaactaaaaacagccatgcagcacttgtaatatttattcaaactgtggtaaggtttttcgcggatcatcgaattaaacaacatacttcattactgatctcagtaacggtctaatgatttcagtttatatgttgccatattactcttgaggtggaatgcttacactttcatttataggctaaatttattatctatctagcctatggcactcatcattgtctgcttggactactagggtatctaatcctaattgatacccaagccttcgtccctcaacgtcagtttttacatagaaggatgccttcgccgttaccagtctctccggtattaaaatatgcaatcactactccagaaattcttccttctcttataaaactctagtaaaaaaacactgttttagtattttatttaccgtctaggtaccctttaaacctaataaagatgaataacactagtcttatacgttttaccgcgactgctggcacgtattttggtcaagacttataaatagaatagttgtcattatctctattctatttagaattttatacgaattaatcgttattgtattattatacattttcattcttccaagttactggttcagcctttcggccattgaccaatattcctcactgctgtacaaaaacgcattggggttttttcagacccaatgtggtcgatcgacctctcagtcacgactacggatattagctagaataagtaattacctttcctactactcaccgtgataaaaattaacatcttaaagcagaccttatattcctttcttttataagggatcttatccccttactttaaggtagccaatttatctttactcacctgtacaccacctacttattagttttttttactaattagtcgttcgattagcatgtgtcaagttcttggacagcgttcaatcagagccatcatcaagctcaac

SEQ ID NO: 5 - DNA, 2103 bp, Unknown
  Newly identified micro-organism
ctaaagtaagcttcgcgcttaaaatgctttcagcacttatctttaactgatgtagctttcctgccatgcctatgaaaacaatttatttaagtattaataaaccatatattaataattaattaatatataacataaacaacaggtaaaccatagatcaacatacccaactcctttcgtacgaaggggctatctttattatactttaatttcctctagaagatagaaaccatactgtctcacgacgtattaaacccagctcatgtaactctttaatcgacgaacagtcgaacccttcatgatttttgcattcatgtggatgagttaagccgacatcgaggtgccaaaccgcgcactcaatttgtactctcttgcgcagattagcctgttcaattttttgttattctaaatttccatttctctcaaaatggttcagactatttcatcatctttactaactatttttaagcaaaaaataaataataattaactaccacttaatcaacctttaattccaaaagatccactacgaaatttagaatttaaattagtatagtttaaattaggttttaagttacctcttaatactgagggattataacccatcatataagaatatacattatctagatttcctttatattttaatttttgttgagattttgaagcagaactacgtttagttaatctacctgcagcttctactctaacacctgatactcttttatatttaatattagataatacaatttttttcagatattttgaacttgttttattttgttctattaaatcatttaataaagtatttgtaatatccttatcattatcatttacagtaaataaactatctaaatcaaaaaaatattttggtctttttattttaatatttttaatttttactttatcgactaaaattgtaagatattttaatactttagttatttttctttttcttaattttaatattaaagattctgtaaatatatcactattaaagaaaaaatattttaaattaataatattaaactctactttttttttatatattttttttattaaactaattaaaccttgtaaatataaattatcaaatttagctttattaatataaagtaattgtttaaaatacatgtaatattttaatcttataagtgatttatttataaaatatttataataaagattttgtactaaagatacttttgaactataattaggtaaaacatttattattattttaccttttttttcttgttgttttataatattcaatcctacatttcttattaattttaatttttttaataatttacgatttttaaataatcttttatatttttttactatttttaataagtaatttaatctttgtctattatatatatataatgttatatttactttatcattagtatgtttaaattcaccatcactaacaaatattttatttatagataattttcttaatctatgacgtaatatttttattttttttcttaatttatattctatatttaaattatatgaatttaaataacctttaattaatttaagtacaaatctgctagcaataggtattaaatttaaagcatttttattataaacataaatactattatttcaatctcttacagcaggaacaaaatctttattataaatagtaacttttggattatttaatgatttttttttatatgtattttttaattttgattttataatatttaacatatttatatataatattaaagtttagctaaaatagctaaatctatttcattattataattaaagtaataataattattatacaaaattattatagttagtaaaaatgttgggttaattattaaagtctagtcgttgaacggctttatttgctacaataaaatccgcttcaaattcacagaggggaaaccctcagttgtctttgaaatttacccaattacaccaatattttacaatattgggggactaacatccctagcgtaactttttcaaaaatccaagaccattccttaatgcatcttgtgatcatatgccccgcttacgcgactgatagatttgtagatcaaacagtaaagcaagatttagccattaaac

SEQ ID NO: 6 - DNA, 492 bp, Unknown
  Newly identified micro-organism
cagtaaagctgcatagggtcttctcgtctatctagaggtaaacagtatctgcactgctattccaatttcactgagacaatcatcgagacagctgttgtatcgttacatcattcatgcaggaccgcatttaacggccaaggtatttcgctaccttaggaccctcatagataaggccgccattaattggggtatccttcaaaacctaagctaaaaacctaggtaaatccgttatccttccaacattagggcagatatcacactcaatactttgatattttatctttgcagagtgctgtgtttttattaaacagtcgtacaacattatttcatgtttcctcttttcattaatctaatttaatgctttaaatttatgaaaatggccctccttattccaaagttacggagtcaatttgccgagttccttaatgattgttctctcaaacgcctttgtattctctacttgcttacttgtgatagtatctaggtacggtt

SEQ ID NO: 7 - DNA, 747 bp, Unknown
  Newly identified micro-organism
aaagtttcggtatattgtttagatccgttaaattttcggtgtttttttctaagtttaatcagtgctctgttacgaggtcttcaaaaaatggccgcttctaagcctatttcctgattgtttaaaaaaaaaagcatccttaatttcacttaacaataattttggaaccttaacctttgttctgggctgtttccctttagacatacaaccttatcgcaatatgtccgattattcaacatacatctttgccatttcgagtcgatcactctccgataaagtcactacaaccccccgatataaacaaaatattgttcgagatcacagttctgtacctgctaagatgttaattaaattacctacttatataggtttcgcggaaaaccagctatactagtcagttttgtctttcactaacttaccacaattcttcggatatctatacaacgataacccgttcggacttttataatcctgaccatggtaagatcactagctttcgggtctaattctagatactcattcattttttcataattggtttatctaagctagtttaatacattaaacatcgcttgcatctaaaattaacttgctgacccattatgcaaaaggtacgctcttattatttacttaaatttaactaaagctgcttataaaactactatttcaaattttacctcacggcactttttcactatcgcttatatactatatttagccttagaggaaggttcccctttattcaaacag

SEQ ID NO: 8 - DNA, 115 bp, Unknown; identical to SEQ ID NO: 1
  Newly identified micro-organism

SEQ ID NO: 9 - DNA, 115 bp, Unknown; identical to SEQ ID NO: 2
  Newly identified micro-organism

SEQ ID NO: 10 - DNA, 115 bp, Unknown
  Newly identified micro-organism
tacgaccatagggtgtggagaacagggcttcccgtccgctcagccgtacttaagccacacgccggccggttagtagttgggtgggtgaccaccagcgaatcccggctgttgtatg

SEQ ID NO: 11 - DNA, 115 bp, Unknown
  Newly identified micro-organism
tacgaccatagggtgtggaaagcagggcttcccgtccgctcagccgtacttaagccacacgccggccggttagtagttgggtgggtgaccaccagcgaatcccggctgttgtatg

SEQ ID NO: 12 - DNA, 115 bp, Unknown; identical to SEQ ID NO: 11
  Newly identified micro-organism

SEQ ID NO: 13 - DNA, 115 bp, Unknown; identical to SEQ ID NO: 2
  Newly identified micro-organism

SEQ ID NO: 14 - DNA, 443 bp, Unknown
  Newly identified micro-organism
tctggttgattctgccagtagtcatatgcttgtctcaaagattaagccatgcatgtctaagtataagcactttatacggtgaaactgcgaatggctcattaaatcagttatcgtttatttgatagtgccttactacatggatacctgtggtaattctagagctaatacatgctgaaaaccccgacttcggaaggggtgtatttattagataaaaaaccaacgcccttcggggctccttggtgaatcatgataacttaacgaatcgcatggccttgcgccggcgatggttcattcaaatttctgccctatcaactttcgatggtaggatagtggcctaccatggtggcaacgggtaacggggaattagggttcgattccggagagggagcctgagaaacggctaccacatccaaggaaggcagcaggcgcgcaaattacccaat

SEQ ID NO: 15 - DNA, 296 bp, Unknown
  Newly identified micro-organism
agtcgggggcgtcagtattcagctgtcagaggtgaaattcttggatttgctgaagactaactactgcgaaagcattcgccaaggatgttttcattaatcagggaacgaaagttaggggatcgaagacgatcagataccgtcgtagtcttaaccataaactatgccgactagggatcggacggtgtttctatgatgacccgttcggcaccttacgagaaatcaaagtttttgggttctggggggagtatggtcgcaaggctgaaacttaaagaaattgacggaagggcaccacaagg

SEQ ID NO: 16 - DNA, 638 bp, Unknown
  Newly identified micro-organism
cacgggagcctgcggcttaatttgactcaacacggggaaactcaccaggtccagacaaaataaggattgacagattgagagctctttcttgatcttttggatggtggtgcatggccgttcttagttggtggagtgatttgtctgcttaattgcgataacgaacgagacctcggcccttaaatagcccgacccgcgttcgcgggccgctggcttcttagggggactatcggctcaagccgatggaagtgcgcggcaataacaggtctgtgatgcccttagatgttctgggccgcacgcgcgctacactgacagggccagcgagtacatcaccttggccgagaggcccgggtaatcttgttaaaccctgtcgtgctggggatagagcattgcaattattgctcttcaacgaggaatgcctagtaggcacgagtcatcagctcgtgccgattacgtccctgccctttgtacacaccgcccgtcgctactaccgattgaatggctcggtgaggccttcggactggcccaggggggttggaaacgaccccccagggccggaaagttggtcaaacccggtcatttagaggaagtaaaagtcgtaacaaggtttccgtaggtgaacctgcggaaggatcattacc

SEQ ID NO: 17 - DNA, 4960 bp, Unknown
  Newly identified micro-organism
aaaactttcaacaacggatctcttggttccggcatcgatgaagaacgcagcgaactgcgataagtagtgtgaattgcagaattcagtgaatcatcgagtctttgaacgcacattgcgccccctggcattccggggggcatgcctgtccgagcgtcattgctaccctcaagcgcggcttgtgtgttgggccgtcgtcccccccggtgcttccggcgggggacgggcccgaaaggcagtggcggcaccgcgaccggtcctcgagcgtatggggctctgtcacccgctccgtgggaccggccggcgccagccctccaaatatgtatatatatatatatacataccaagttgacctcggatcaggtagggatacccgctgaacttaagcatatcaataagcggaggaaaagaaaccaaccgggattgccctagtaacggcgagtgaagcggcaagagctcaaatttgaaatctggcccctccggggtccgagttgtaatttgtagaggatgcttcgggtgcggcccccgtcgaagtgccctggaacgggccgtcggagagggtgagaatcccgtctgggatggggtgcccgcgcccgtgtgaagctccctcgacgagtcgagttgtttgggaatgcagctctaagtgggtggtaaatttcatctaaagctaaataccggccggagaccgatagcgcacaagtagagtgatcgaaagatgaaaagcaccttgaaaagggagtgaaacagcacgtgaaattgttgaaagggaagcgctggcgaccagactcgcccgcggggttcagccggcattcgtgccggtgtacttccccgtgggcgggccagcgtcggtttgggcggccggtcaaaggcccccggaatgtagcgcctctcggggcgccttatagccgggggtgcaatgcggccagcccggaccgaggaacgcgcttcggcacggacgctggcataatggtcgtcaacgacccgtcttgaaacacggaccaaggagtctaacatctacgcgagtgctcgggtggcaaacccgtgcgcgcagtgaaagcgaacggaggtaggagcccccccgtggggcgcactatcgaccgatcctgatgtcttcggatggatttgagtaggagcgtagctgtggggacccgaaagatggtgaactatgcctgaatagggtgaagccaggggaaactctggtggaggctcgcagcggttctgacgtgcaaatcgatcgtcaaatttgggtataggggcgaaagactaatcgaaccatctagtagctggttcctgccgaagtttccctcaggatagcagtaacgcggatcagttttatgaggtaaagcgaatgattagaggccttggggttgaaacaaccttaacctattctcaaactttaaatatgtaagaagcccttgtttcttcagtgaacgcgggcattcgaatggtgcgttactagtgggccatttttggtaagcagaactggcgatgcgggatgaaccgaacgcgaggttaaggtgccggaatgcacgctcatcagacaccacaaaaggtgttagttcatctagacagcccgacggtggccatggaagtcggaatccgctaaggagtgtgtaacaactcacgggccgaatgaactagccctgaaaatggatggcgctcaagcgtgctaccgatacctcgccgccggggtagaagcgacgccccggcgagtaggcaggcgtgggggtccgtgacgaagcccagggagtgatcccgggtcgaacggcccctagtgcagatcttggtggtagtagcaaatactcaaatgagaactttgaggactgaagtggggaaaggttccatgtgaacagcaattggacatgggttagtcgatcctaaggcatagggaagttccgtttgaaaggcgccctgcgcgccgtgtgccgaaagggaagccggttaacattccggcacctggatgtggattctccacggcaacgtaactgaacgcggagacgtcggcgggggccctgggaagagttctcttttcttcttgacggcctatcaccctgaaatcggtttgtccggagctagggttcaacggccggcagagccccgcacctttgcggggtccggtgcgcccccgacgacccttgaaaatccgcgggaaggaatagttttcacgccaggtcgtactcataaccgcagcaggtctccaaggtgaacagcctctagttgatagaacaatgtagataagggaagtcggcaaaatggatccgtaacttcgggataaggattggctctaagggtcgggcccgctgggccttggggggaaccccccggagcaggggggcactagccgggcaaccggccggcgccccccagcaccgggcgggggacgcccttggcaggcttcggccgtccggcgggcgcttaacgaccaacttagaactggtacggacaaggggaatctgactgtctaattaaaacatagcattgcgatggccagaaagtggtgttgacgcaatgtgatttctgcccagtgctctgaatgtcaaagtgaagaaattcaaccaagcgcgggtaaacggcgggagtaactatgactcgagaatcacgtggacgaacgatggctaccacagtgagagggtcaagcggcgtgaggagaagacgtcgctagtgagggggggaggagcacggaggggcggtcccggcccggcgtgcctcgtgtccccttgcgacaccgtcaaattgcgggaacttcctaaagcctctgccaccgcggctcgccgaaaggcgcagtgcagcaccagggtaatgacctcggggatggtaatagcgcagaggatgtgccaatggatgatccgcagccaaaccctacgtcccccccgctccagggggggatacgggcgcagtccaacgactagatggcggtgggtctcccggggaaggccccggggggtctaagatatagtctgacggtccgccgaaaggcgtgtgtggccgcagaatgctcttaaggtagccaaatgcctcgtcatctaattagtgacgcgcatgaatggattaacgagattcccactgtccctatctactatctagcgaaaccacagccaagggaacgggcttggcaaaatcagcggggaaagaagaccctgttgagcttgactctagtttgacattgtgaaaagacatatggggtgtagaataggtgggagcttcggcgccggtgaaataccactacctttatcgtttttttacttattcaatgaagcggaactgggcttcaccgcccatcttctggcgttaaggtccttcgcgggccgatccgggttgaagacattgtcaggtggggagtttggctggggcggcacatctgttaaaccacaacgcaggtgtcctaagggggactcatcgcgaacagaaatcgcgagtggagcaaaagggcaaaagtccccttgattttgattttcagtgtgaatacaaaccatgaaagtgtggcctatcgatcctttatgtccctcgaaatttgaggctagaggtgccagaaaagttaccacagggattaactagatatagtcccaggccccgacgcctggttggggtctagtccggctgccgtcgagactgtgcgggtggcagctaagaaagtcccggtcgtccgggcctttctgtagggcaacacatctggatgcggggaactctcgccaggtctctagtaccaggtggccgggtaacgcccggtcacggagtctgttcagggcagacgggtaaaaacctagggaatagagacaatccgcagccgacccggctccctgccccccttccgtcggggcaccagctgggcggttcaacgctcggtaagatgtgggtgcgccccccctggggggcgcgcttaaggtacgggctacgcccacccgagagggtgcggccgcctaccgaccggcatagggtcgagaagcggccggtgcgggctcaccggtgatgcgtcctgcctgccccccttgtccgggggggccaggaccccggagggcccgctggtagtacggaactggcttgtggcagccaagcgttcatagcgacgttgctttttgatccttcgatgtcggctcttcctatcataccgaagcagaattcggtaagcgttggattgttcacccactaaaccatcgagaacgtatagttccccattggtggggatagccgggcctccgcgagggcgcgggggttaggccggctagtcgatacagcaggaccgctgcaggtgctgtacggcgacacaacctggatcgggggaggctgccgggggccacggagcgccgtggtcgccatgctaatcccgagccgagccgcggtggagcgatccgccgtcgaggccggtgtagagcgcggaaaggtgtgggtggcgctgggggtcagacctcaggccgcttaagggacgtgccaacccctagggaaacctagcccgagtgcgaaggtcctgcaggccggatcacacggggggcagtgagccgcggaggaaatgccgtggggagcctggtatgggcgggggaggtggatcgacacccccccgaccccatcgtgaatagggaacgtgagctgggtttagaccgtcgtgagacaggttagttttaccctactgatgaaggtcgccgcaacggtaattcaatttagtacgagaggaaccgttgattcagataattggtttttgcggctgtctgatcaggcagtgccgcgacgctaccatctgccggataatggctgaacgcctctaagtcagaatccgtgccggaacgcggcgatatcgccccgcacgtcgtagttggatacgaataggcctccgggccatggacctcagcaggctggcgacggttcccggggagaagcccccgggagccagctggcggattgcaatgtcacctcgcgcggggatagatcctctgcagacgactgaagtgaccaagcgggtcgtgtaagcgct

SEQ ID NO: 18 - DNA, 115 bp, Unknown; identical to SEQ ID NO: 1
  Newly identified micro-organism

SEQ ID NO: 19 - DNA, 84 bp, Unknown
  Newly identified micro-organism
cttctcgatggtccagtggtcaagatacccgcttgtcattcgacaagccgcgggtgaccggggttcgattccccgtcgggaagt

SEQ ID NO: 20 - DNA, 72 bp, Unknown
  Newly identified micro-organism
tccaatgtggtctaacggctaggataccgagctttcacctcggaggtcggggttcgattccccgcattggaa

SEQ ID NO: 21 - DNA, 83 bp, Unknown
  Newly identified micro-organism
tggcaagatggccgagcggttaaggcgcatgtttcaggtacatgttctgcaaagatcgtgggttcgaatcccactcttgtcat

SEQ ID NO: 22 - DNA, 83 bp, Unknown
  Newly identified micro-organism
gacctgctggtgtagtggttatcacgcaatgctcacatgaattgtgccattgaggtgctcggttcgatcccgaggtaggtcac

SEQ ID NO: 23 - DNA, 74 bp, Unknown
  Newly identified micro-organism
taggtgattagtttagtggcagaacgtgtcgtttacaccgacaaggtcgacggttcgatcccgtcatcacctaa

SEQ ID NO: 24 - DNA, 74 bp, Unknown
  Newly identified micro-organism
agtcctttaggatagctggttattccgcatcgttaacaccgatgaggtcggcggttcgaacccgtcaaggacta

SEQ ID NO: 25 - DNA, 74 bp, Unknown; identical to SEQ ID NO: 24
  Newly identified micro-organism

SEQ ID NO: 26 - DNA, 88 bp, Unknown
  Newly identified micro-organism
gggcttgtggtctagtggtatgacgcgtcattcgcatattctgcaatggaaattgatgaggtccagggttcaattccctgcaagtcca

SEQ ID NO: 27 - DNA, 81 bp, Unknown
  Newly identified micro-organism
ggccggctggcctaatggttaaggcttcactctcctactctggttaagtgaggattgcgggttcgaatcccgtgtcggtcg

SEQ ID NO: 28 - DNA, 72 bp, Unknown
  Newly identified micro-organism
gcatcattggttcagtggtagaattcctgacttccaatcagatgacccgcgttcgattcgcggatgatgcac

SEQ ID NO: 29 - DNA, 83 bp, Unknown
  Newly identified micro-organism
tggcaggatggccgagcggttaaggcgcagcattagaaatgctgttctttcgagatcgtgggttcgaatcccactcctgtcga

SEQ ID NO: 30 - DNA, 83 bp, Unknown
  Newly identified micro-organism
tggcgagatggccgagcggttaaggcgctagagtaaggttctagtatcgaaagatgcatgggttcgaatcccattctcgtcat

SEQ ID NO: 31 - DNA, 72 bp, Unknown
  Newly identified micro-organism
agcatggtagctcaggggaagagcgccgggctcataacccggaggtccctggatcgaaaccaggccatgcta

SEQ ID NO: 32 - DNA, 81 bp, Unknown
  Newly identified micro-organism
ggcgagatggccgagcggttaaggcgctagagtaaggttctagtatcgaaaggtgcatgggttcgaatcccattctcgtca

SEQ ID NO: 33 - DNA, 72 bp, Unknown
  Newly identified micro-organism
tccggtatggtgtagtggttaacatcgccgtctctcacacggcagccgggggttcgattccccctaccggaa

SEQ ID NO: 34 - DNA, 88 bp, Unknown
  Newly identified micro-organism
agccctcgtggcctaactggttaaggcgtaaggcttctatttattaaggcgaccttaagattgcgggttcgagtcccgccgggggttt

SEQ ID NO: 35 - DNA, 72 bp, Unknown; identical to SEQ ID NO: 33
  Newly identified micro-organism

SEQ ID NO: 36 - DNA, 81 bp, Unknown
  Newly identified micro-organism
ttctcgatggtccagtggtcaagatacccgcttgtcattgacaaatcgcgggtgaccggggttcgattccccgtcgggaag

SEQ ID NO: 37 - DNA, 87 bp, Unknown
  Newly identified micro-organism
ggtcctatggtctaggggttaggacgtcggattttgattattatttccgaacttccgaaagcgagggttcgaatccctctaggacct

SEQ ID NO: 38 - DNA, 71 bp, Unknown
  Newly identified micro-organism
gcccgcttagtctagtggtaagacgtttcactcgtaatgaaaagtggtcagttcgattctggcagtgggca

SEQ ID NO: 39 - DNA, 75 bp, Unknown
  Newly identified micro-organism
aggtcgcgtggctcaattggcagagtgcttgactacgaatcaagaggttcggggttcgaacccccgcgtgacctt

SEQ ID NO: 40 - DNA, 71 bp, Unknown
  Newly identified micro-organism
gcattgttggtctagtggtagaattcatcgttgccatcgatgaggcccgcgttcgattcgcggacaatgca

SEQ ID NO: 41 - DNA, 71 bp, Unknown; identical to SEQ ID NO: 40
  Newly identified micro-organism

SEQ ID NO: 42 - DNA, 75 bp, Unknown
  Newly identified micro-organism
tgcattgttggtctagtggtagaattcatcgttgccatcgatgaggcccgcgttcgattcgcggacaatgcatcc

SEQ ID NO: 43 - DNA, 71 bp, Unknown; identical to SEQ ID NO: 40
  Newly identified micro-organism

SEQ ID NO: 44 - DNA, 104 bp, Unknown
  Newly identified micro-organism
tgactttgctggcgtagtggacgcgacatcttcgtgactcgagttcacggatggcgatatagattgccgggtgttattctgttcctctctcggagaagggtcgg

SEQ ID NO: 45 - DNA, 87 bp, Unknown
  Newly identified micro-organism
ggtcctgtagctcaatggtgagagtttcaagcttatgggcatggttacattccttgacggttgtgggttcgagtcccaccgggacca

SEQ ID NO: 46 - DNA, 90 bp, Unknown
  Newly identified micro-organism
ggaagcctggatgaggagcgccctagaatctgttggattctatgttgagcacatagagacagagtatcgtcccacgcgactgacctccac

SEQ ID NO: 47 - DNA, 81 bp, Unknown
  Newly identified micro-organism
tgcattgatggtgtagtggtatcacaccgaccttccataccgagagtcggtaaccggggttcgattccccgtcaacgcatc

SEQ ID NO: 48 - DNA, 73 bp, Unknown
  Newly identified micro-organism
gtcctcgtggcccagcggttaaggcgctcggctgttaaccgagagatcggaggttcgatccctcccgtggacg

SEQ ID NO: 49 - DNA, 81 bp, Unknown
  Newly identified micro-organism
aggttgtatggtctagtggttatgacgtgtgactctgatgtggaatcacatagccttggttcgattccgagtacgacctac

SEQ ID NO: 50 - DNA, 73 bp, Unknown
  Newly identified micro-organism
ggtcgtatggtctagtggttatgacgtgtgactctgaatcacatagccttggttcgattccgagtacgacctc

SEQ ID NO: 51 - DNA, 85 bp, Unknown
  Newly identified micro-organism
gcgccgatggtcaagtggttacgatgtggtcctcccattctgtgaggttagaccgagacccgagttcgaatcccggtcggcgcac

SEQ ID NO: 52 - DNA, 75 bp, Unknown
  Newly identified micro-organism
tggccgtgtggcgcaatggtagcgcgtcggtttccggtaccgaaggcttgcgggttcgaatcccgtcatggtcga

SEQ ID NO: 53 - DNA, 72 bp, Unknown
  Newly identified micro-organism
ggtgctatagtctaacggtcaggacggcacgttgtggccgtgcaggtttgggttcgattcccaatggcgcca

SEQ ID NO: 54 - DNA, 85 bp, Unknown
  Newly identified micro-organism
aggaagggtccgtttgttggttagcgggttgagctgtaaactcaatggctataggccatcgaaggttcgattccttttcttccta

SEQ ID NO: 55 - DNA, 73 bp, Unknown
  Newly identified micro-organism
agctcttatagctcaatggtagagcggaatactgttaatatttttatagatgttcgattcatcttaagggctt

SEQ ID NO: 56 - DNA, 73 bp, Unknown
  Newly identified micro-organism
attcttattagctcaatggtagagcagaatacttctaatattttgatccaagttcgagtcctggataagaata

SEQ ID NO: 57 - DNA, 73 bp, Unknown
  Newly identified micro-organism
aggcatgttaatttaatggaagaatagcgtgctacggacacgaatatataagttcgagtcttatacatgtctt

SEQ ID NO: 58 - DNA, 73 bp, Unknown
  Newly identified micro-organism
ggaaggtatagtttaaaggtagaacagctgtatgtggcacagtaaatcttagttcgattctaggtacctccct

SEQ ID NO: 59 - DNA, 73 bp, Unknown
  Newly identified micro-organism
agccagtgtagtttaatggtagaacaataatttcatgaattaagaatgagaattcgactttctcctctggctt

SEQ ID NO: 60 - DNA, 73 bp, Unknown
  Newly identified micro-organism
tatgttgtagactaatcggtaagtcataaatttttggtatttacttatgggtgttcgagtcgccccaacatag

SEQ ID NO: 61 - DNA, 84 bp, Unknown
  Newly identified micro-organism
atgggtgtgctgaaatttggtaaccaggttctgcttaggacagaatagtttttaactttacaagttcgagtcttgttacccata

SEQ ID NO: 62 - DNA, 75 bp, Unknown
  Newly identified micro-organism
tgcttgagaagctcaattggtagagcggatcactgaagatgattaggttgtaagttcaagtcttgtctcaagcag

SEQ ID NO: 63 - DNA, 74 bp, Unknown
  Newly identified micro-organism
tggggttatagtttaactggtaaaacaacgattttgcatatcgttaattcaggatcgagtcctgataactccaa

SEQ ID NO: 64 - DNA, 82 bp, Unknown
  Newly identified micro-organism
atccgagtgctggaattggtagacagtcttaacttaagattaagtggtgtaagccgtaaacgttcaagtcgtttctcggata

SEQ ID NO: 65 - DNA, 73 bp, Unknown
  Newly identified micro-organism
aaggctatagcttaataggtaaagcgaaccactcatgatggtttgagtaaatgttcaagtcattttagcctta

SEQ ID NO: 66 - DNA, 73 bp, Unknown
  Newly identified micro-organism
aagaaattagctcagttggtagagctgtcgctttacacgcgaaaggtcaggtgttcaagtcacctatttctta

SEQ ID NO: 67 - DNA, 74 bp, Unknown
  Newly identified micro-organism
gacccaatggtcaagtttggttaagacataacattttcactgttagtgcgggagttcaaatctcccttgggttg

SEQ ID NO: 68 - DNA, 75 bp, Unknown
  Newly identified micro-organism
tgccttttttgcataattagataatgcaaccaccttgtaagtggtagatgcaagtgcaattcttgcattaggcat

SEQ ID NO: 69 - DNA, 72 bp, Unknown
  Newly identified micro-organism
caggttagagccaggtggtgaggcaacttatttgggttaagtcttttttatgttcgaatcataataacctga

SEQ ID NO: 70 - DNA, 86 bp, Unknown
  Newly identified micro-organism
agagagttggctgagtggtttaaagcggttagcttgagtctaactaaaggtaaaacctttcatatgttcgaatcatatactctctg

SEQ ID NO: 71 - DNA, 74 bp, Unknown
  Newly identified micro-organism
tgattctttaacttaataggtaaagtgtgttcttgataaggatatgttcagtgttcgattcactgaagaatcat

SEQ ID NO: 72 - DNA, 72 bp, Unknown
  Newly identified micro-organism
aagagcatagtttaataggcaaaactgtaagcttcaaccttatatttcttagttcaagtctaagtgctcttg

SEQ ID NO: 73 - DNA, 81 bp, Unknown
  Newly identified micro-organism
ggaaaagtttccaagggtagggtaagatatttgctaaatattgtgtttttacacttagatgttcgattcatctcttttccg

SEQ ID NO: 74 - DNA, 73 bp, Unknown
  Newly identified micro-organism
gggttagtaacttaataggtaaaggattttcttgtcgagaaagtagatgccggatcgaaaccggtctaactcg

SEQ ID NO: 75 - DNA, 72 bp, Unknown
  Newly identified micro-organism
atggctatatgtcaattggtagacatgttatcttccacataacaagtgtcgattcgagttcgactagccata

SEQ ID NO: 76 - DNA, 71 bp, Unknown
  Newly identified micro-organism
atgactataagttaacggtagactacttatttaccaaataagatgtgctgattcgaattcagctagtcata

SEQ ID NO: 77 - DNA, 72 bp, Unknown
  Newly identified micro-organism
gagactttagtttaataggcaaaaccaatgacttttaatcattttttatgggttcaagtcccataagtctta

SEQ ID NO: 78 - DNA, 90 bp, Unknown
  Newly identified micro-organism
actgggggagtcgcgaggggaagggcggacaggtcttcggggcccgtgcggatggagctgatgggctgggttctatgcctgtccccggtg

SEQ ID NO: 79 - DNA, 82 bp, Unknown
  Newly identified micro-organism
gggtttgtggtccagtggtacgatgcatgcttcgggaagactgatatgtatgcgacccgggttcgactcccggcaaaccccc

SEQ ID NO: 80 - DNA, 75 bp, Unknown
  Newly identified micro-organism
tgggcttgtagctcagttggtagagcgttcgctttgcatgcgaaaagtctgggtttcgaatacccacaagtccat

SEQ ID NO: 81 - DNA, 88 bp, Unknown
  Newly identified micro-organism
gcctggatagttcagtggcagaattcatcgtttgggtatagctttgctcatctcgatgaggtcctgggttcgatccccagttcaggcc

SEQ ID NO: 82 - DNA, 87 bp, Unknown
  Newly identified micro-organism
tggcaagatggcggagtggttaacgcgttgcactcgaatgctatgcaatcccttcgggggcctgagttcgaatctcagtcttgtcga

SEQ ID NO: 83 - DNA, 75 bp, Unknown
  Newly identified micro-organism
tgtcctcgtggcccagcggttaaggcgctcggctgttaaccgagagatcggaggttcgatccctcccgtggacgt

SEQ ID NO: 84 - DNA, 82 bp, Unknown
  Newly identified micro-organism
ttctcgatggtccagtggtcaagatacccgcttgtcattcgacaagccgcgggtgaccggggttcgattccccgtcgggaag

SEQ ID NO: 85 - DNA, 76 bp, Unknown
  Newly identified micro-organism
tggtcgcgtagctcagttggttagagcgcgacactaataatgtcgaggccgtgggttcgagcccctccgtgaccat

SEQ ID NO: 86 - DNA, 76 bp, Unknown; identical to SEQ ID NO: 85
  Newly identified micro-organism

SEQ ID NO: 87 - DNA, 89 bp, Unknown
  Newly identified micro-organism
ggaagaatggcagagtggtaatgcaccggcttgctaagccgagataaccagagatggctgcgctggttcgataccagcttcttccgcca

SEQ ID NO: 88 - DNA, 87 bp, Unknown
  Newly identified micro-organism
ggagggttctgctaggttggctggcaagcggtcttgaaaaccgtggcaacggcaacgttgggggttcgactcctcaaccctccgcca

SEQ ID NO: 89 - DNA, 643 bp, Unknown
  Newly identified micro-organism
gtcgtaacaaggtttccgtaggtgaacctgcggaaggatcattaccgagtgcggcacccccccgggggtgccaacctcccacccgtgtctaccgtaccatgttgcttcggcgggcccgcccccccagcaggaggggtcgccgggggggcatctgtcccccccaggtgcgcgcccgccggagacacccacacgaacgcttgtctgaaggactgtcgtctgagtggattgatcaaatcagttaaaactttcaacaacggatctcttggttccggcatcgatgaagaacgcagcgaactgcgataagtagtgtgaattgcagaattcagtgaatcatcgagtctttgaacgcacattgcgccccctggcattccggggggcatgcctgtccgagcgtcattgctaccctcaagcgcggcttgtgtgttgggccgtcgtcccccccggtgcttccggcgggggacgggcccgaaaggcagtggcggcaccgcgaccggtcctcgagcgtatggggctctgtcacccgctccgtgggaccggccggcgccagccctccaaatatgtatatatatatatatacataccaagttgacctcggatcaggtagggatacccgctgaacttaagcatatcaataagcggagga

SEQ ID NO: 90 - DNA, 940 bp, Unknown
  Newly identified micro-organism
acccgctgaacttaagcatatcaataagcggaggaaaagaaaccaaccgggattgccctagtaacggcgagtgaagcggcaagagctcaaatttgaaatctggcccctccggggtccgagttgtaatttgtagaggatgcttcgggtgcggcccccgtcgaagtgccctggaacgggccgtcggagagggtgagaatcccgtctgggatggggtgcccgcgcccgtgtgaagctccctcgacgagtcgagttgtttgggaatgcagctctaagtgggtggtaaatttcatctaaagctaaataccggccggagaccgatagcgcacaagtagagtgatcgaaagatgaaaagcaccttgaaaagggagtgaaacagcacgtgaaattgttgaaagggaagcgctggcgaccagactcgcccgcggggttcagccggcattcgtgccggtgtacttccccgtgggcgggccagcgtcggtttgggcggccggtcaaaggcccccggaatgtagcgcctctcggggcgccttatagccgggggtgcaatgcggccagcccggaccgaggaacgcgcttcggcacggacgctggcataatggtcgtcaacgacccgtcttgaaacacggaccaaggagtctaacatctacgcgagtgctcgggtggcaaacccgtgcgcgcagtgaaagcgaacggaggtaggagcccccccgtggggcgcactatcgaccgatcctgatgtcttcggatggatttgagtaggagcgtagctgtggggacccgaaagatggtgaactatgcctgaatagggtgaagccaggggaaactctggtggaggctcgcagcggttctgacgtgcaaatcgatcgtcaaatttgggtataggggcgaaagactaatcgaaccatctagtagctggttcctgccgaagtttccctcagga

SEQ ID NO: 91 - DNA, 1533 bp, Unknown
  Newly identified micro-organism
gtagtcatatgcttgtctcaaagattaagccatgcatgtctaagtataagcactttatacggtgaaactgcgaatggctcattaaatcagttatcgtttatttgatagtgccttactacatggatacctgtggtaattctagagctaatacatgctgaaaaccccgacttcggaaggggtgtatttattagataaaaaaccaacgcccttcggggctccttggtgaatcatgataacttaacgaatcgcatggccttgcgccggcgatggttcattcaaatttctgccctatcaactttcgatggtaggatagtggcctaccatggtggcaacgggtaacggggaattagggttcgattccggagagggagcctgagaaacggctaccacatccaaggaaggcagcaggcgcgcaaattacccaatcccgacacggggaggtagtgacaataaatactgatacggggctcttttgggtctcgtaattggaatgagagcaatttaaacccctcatcgaggaacaattggagggcaagtctggtgaaccatcagttctacaatgctgacgccagagatagtaggaccctccctcccggggagggttacgcctactagtcgagcactcgcaatagcgatgggtgagtgccggcgaggtgacctggtacgggggagcctaagggtgcggcctggaagagaggtcgacgacacctatggtaatcccgtggcgagcctacacggccgtcgtaacgcgcggaaaggcaccggtcgctagagatctagcggctcaagggacgtgctgtcccatccgaaaggatgcctgcaactggagcacccatcgtgtaaaggttgtggggggtttgcagcgggccgctgtaagcctgggggtctctcatcgtggcatggcgaggaacgtcgccacgtcgatgaatgagagcgaaaacggccagcagccgcggtaattccagctccaatagcgtatattaaagttgttgcagttaaaaagctcgtagttgaaccttgggcctggctggccggtccgcctcaccgcgagtactggtccggctgggcctttccttctggggaaccccatggccttcactggccgtggggggaaccaggacttttactgtgaaaaaattagagtgttcaaagcaggcctttgctcgaatacattagcatggaataatagaataggacgtgcggttctattttgttggtttctaggaccgccgtaatgattaatagggatagtcgggggcgtcagtattcagctgtcagaggtgaaattcttggatttgctgaagactaactactgcgaaagcattcgccaaggatgttttcattaatcagggaacgaaagttaggggatcgaagacgatcagataccgtcgtagtcttaaccataaactatgccgactagggatcggacggtgtttctatgatgacccgttcggcaccttacgagaaatcaaagtttttgggttctggggggagtatggtcgcaaggctgaaacttaaagaaattgacggaag

SEQ ID NO: 92 - DNA, 8811 bp, Unknown
  Newly identified micro-organism
atgtcgaacgtctactttccctactcaaaagcgcctctgcgcaccataaaggagatccagtttggtctgttttctcccgaggaggtgaagaggatgagcgtggtccacgtggaatacccggagacgatggtctgtgtccttacgcggaccggtcaggatggaagatgtgctgacaaggtcaacaggacgaccagagggtgcgacctcgggccaaaggtttgaatgatccgcgcctaggaacgatcgatcgtcagtggaactgcgagacttgcgaggaaggccagagagaatgccccgggcactttggccatatcgaactggcaaccccggtcttccacatcggtatgccggatactctactgtctacttgacaaattactgacactttgtctaggctttttgacgaaggtcaaaaaactgttggagactgtctgccataactgtggaaagatcaaagccaacacggttagtcatcccttatgggatggcaaatcttatatggcaatttgtgctgacactggaccagtccgatccaaagtttttagaagccatccgcatgagagatccgaagaggcgtttcgacagcatttggcggctctcgaaagacgttttgatctgtgaagccgacccatcgcctgatgatgatgaacctttttcaaaagagagctccaaaccaatccggacacatggcgggtgtggcaatgcccagcctgtgattcgcaaggaggggatttccttgaccgggacatggaagcctaataagagcttgatggatgagatggagatacagcagcccgaaaagaaaaccattactccgcagatggccctcaatgttttccggaacatttctcatgaggatgtgcgcatcatgggcttgagtaatgattacgctcgccctgagtggatgatcatcactgtcctgccggttcctcccccaccagttcgcccgagtgtccttgtcgggggtagctccagtggccagcgcggtgaggatgacttgacgtacaaacttgcagaaattatccgtgcaaatcagaacgtgcaacgctgtgagcaagaaggtgcccctgagcacgtgattcgcgaattcgaatctttgctgcagtatcacgtcgccacttacatggataatgatattgctggccagccaaaggctatgcagaagtccaacagaccggttaaggcgcttcgctcccgtctgaagggtaaggagggccgtctgcggcaaaacttgatgggaaaacgtgtggacttttccgcgcgtactgtgattacgggcgaccctaatatctccctcgacgaagtcggcgttccgaggagcattgctaggtcactgacctatcctgaagttgttacgccttacaacatcgataaattgcagatgttaatcatgaatggtccaaatgcgcatcctggagcgcgatatattgtcagagacaatggcgaacgtatcgatttgcgtcatgcgaaaagagccggcggtcagcagttgctctatggttggaaggtcgagcgtcatcttatggatggtgatgtgatcctgttcaaccggcagccatctctgcacaaggaatccatgatgggccaccgtgtccgtgtgatgtcatattcaacgttccggttgaatctttctgttactactccgtacaatgctgacttcgatggcgacgagatgaacctccacgttccgcagggcgaggaagcccgggcagagctcgatcaacttgcaatggttcctttgaacatcgtgtctccccagcggaacggcccactcatgggtattgtgcaagacacgctttgtggtatctataaaatttgccgacgcgatacctacctaaccagggaacaagtgatgaacatcatgctttgggtacctgactgggacggtgtcattcctcccccagccatcgtgaaacctaggccaagatggactggaaagcagatgatcagtatggctcttccatctggcctcaatctgctacgtgttgagaaagacagctcgactctttctgaaaagttctccccactaaatgatgatggcctacttatccacggcggacagttgatgtatgggatgttttccaagaaaactgttggcgctactggtgggggtgtcatccatatcatttttaatgaatatggagcagatgctgccgtcgctttcttcaatggcgcccagaccattgtcaattattggctgctgcataatggcttcagtatcggaattggtgacacgattccggaccctgtaacaattcagaggattgaagaatgcgttcgcaatcgcaagaaggaggttgaatccattacgttaagcgcaactgacaataccctcgaagcgctgcctggtatgaacgtgcgagagacgtttgagagtaaggtcgcgcgcgcgctcaacaatgcacgtgatgaagctggtggtgagaccgagaagagtttgaaggatagtaaccacgctatccaaatggctcgttctggatcaaagggctcgaccatcaatatttctcagatgactgcggtcgttggacagcagtctgtggagggcaagcgtattccctttggattcaagtatcgtactctaccgcacttcaccaaggatgactattccccggagtctcgtggttttgttgaaaactcttacctgcgcggattgacccctaccgaattctttttccacgcaatggctggcagggagggtctcatcgatactgctgtgaaaacggccgaaaccggttatattcagcgaaagcttgtcaaggcccttgaagaggttatggtcaagtacgatggcacagttcgcaactcactgggggatatcatccagtttatctacggagaagacggcctcgacggtgctcatattgagaaccagcgggtggacatcatcaggtgctctgataacaaattcatggaccgtttccgtatcgacgtcatggatcctgagcggagcctgggccctgaagtattggaacaggccaacgagattgccggtgacatggaggttcagcgataccttgatgaagagtgggagcaactcctcaaggaccgcgctttccttcgttccgtcgccaaggaagatgaggagatgatgcagctcccaatcaacgttcagaggatcctcgagtcggccaggactacttttaggatccgtgagggcactatcagtgatttgcatccagcggaagttattcctcaagtccaaggattacttaatcgcctgttggttgtacgcggtgatgaccctatttctcatgaggcacaggaggatgcaactctactgtttaaggcacagctgcgtagccgtcttgcattcaagaggctcgtcactgagtactcattgaacaagctcgcttttcagcatgtcctcggcgctattgaaagccgatttgcgaaagctattgccaaccctggtgagatggtcggagtgctctccgcacaatccattggtgagccagctacgcagatgacactgaacaccttccactttgctggtgtttcgtccaagaacgttacccttggtgttccacgtctcaaagagattctcaatgtggctgcgaacatcaagactccatctatgactgtttaccaggaaccggggagagctcatgacaaagagggcgcgaagcagctgcggagcgctgtcgagcacaccagcttaagatcagtgacggaaagcactgagatctattatgatccggatattcagacgactgtgatcgaaaatgacagggacatggtagaatcttacttcatcattcctgaagatgtcaccgacgattcgactcgccagtcaaagtggctgctgcgtatcgttctcagccgcgcgcaactccttgacaaggggcttacggttcaggatgtcgcttccaagatcaagcaagcgtaccctagggacatcgcagtgatattcagcgacaacaacgccgatgagcaggttatccgtattcgtcagctccaggaccataaggaagatgatgatgatgacgagattgaatacgatgttacactgaagaaactggaggagcacctgcttgataccctcactcttcgcggtgttgacggagttgagcgcgcgttcatcaatgaaaggagcaaggtccgggttctcgaagatggctcccttttctcaagcaagagcgacccgctctgccgagaatgggttctcgagactagtggctcctcccttggcgaagttctgtcagtccctggagtcgacgccacccgcacgtattccaaccagttcattgaagtgttccacgtcttcggcgtcgaagcagctcgtgcggcggtcctccgcgaattgacccaggtccttgcgttcgacggctcctacgttaatcaccgtcaccttgcacttttggtcgacatcatgactgtacggggctatcttacacctgtcactcgccacggtatcaaccgggcagataatggcgcacttatgcgttgttctttcgaagagacggtggagattctgcttgaagcagcggcctttggagagctcgacgactgtcgcggtgtttcggagaatttgatcttgggccagatggcacctgccggtaccggagagtttgatatttacctcgatcagggtatgatgaacacggtcgtatcgaacaatgcgcggttcggtgtgatgggcgcgatcggcgctaaagacgcgatcatcgcggacggtgctgccactcagtatgacactgggtcgccgatgcaggagagtgcttatatcggcacgcccgatcccgactcttccttctcgccgatcggtcaagcgggcgcggaaacccctggtggctttacagaatatcagcctcctggattcggaggtgggttcagtcctgccgccagaagcccaggtggttattcgcccagcagtccgttcaatacgagcccgacatctcctggatattcgccaacatcaagctactcacctacgtcacctggcatggggatcactagccctcgattcatgtcatcgccaggcttctcaccggctagtccgtcatttgctccaacgtctccggcatattcgccaacatcgccaacatcaccttcgtactccccaacatctccagggttctcaccgacttcccccaactacagccctacatcaccgagcttcagtccggcgtctcctgccttcagccccacgtcgcctagttatagcccgacgagcccggccatcggtggagctggggcgaatctgtcacctacctccccaacatcccccaagtacacacccacttcgccaggctggtcccccacaagcccgcagacatactcacctacctcccctaactttgctggctcaccgacttcgcctggtggaccaacttctccaggctacagtccgacttcgccggcttacagtcccacgtgagtcccgccttattgagctctaatgaacttctgtggctgataattcccgccagatctccccgccagtgaagtcagcacctcgtactgtgttacggcgaagtttcattacatcgttgtgccacgatcggcctactgagaagaaaccaaaagatacatttcgcatcttacgttgtaaaattggttggttatttcgttcacatcctggccaactgcagcctattcctgatgtatcctcctctcatgaaccagccatagtggtttcttctgcttctgcgcgcgccgtgtttaataggtttccggccgaccttcgaagattgcccctggttttgggggtcggtcatggatgttttttcgctgaataccaagcgtcttagaactgaggctttacaggtggtatcgctatcgcaaggactgctggattattattcttattcatgtacacagctagcagcggtatagaaatcaagaggttgctcgatgctcgatgatcagtgctaggtactgtacctaaggtagtctacacagtaaaatagttgttacatactgtgaagttgggctgcgtacggatatctgcacagaccaagtcggcaaaaaagagctccgagagacaggtggcccattccaacttcctacgtatcttcttcaactcccccgcgggtcatgtccgcttgaagtctatggggtcgcgatgctcgtctcactctctacttgcttaatattctcactggcatcaaaatgaagccgtggcactggtgctccctttcattcgcactccgtaagtggcccttccccactgagctgggcttaggtttttttcggagaactgatcttgcaacgttctcagtgctcccgcaggtgctcgctgtccaagaccgaggtccacttgtagatgcagcacatgtttcacaccataatgtccatcatgatgccagatcatcgagtgggaccgaagatggtgatgtttggcatgggaatggtaagggttacccggcttcgctctgaacgaacttcgctccccccaacggatactgataatgcaaccccttccagaacacgtccaaaaggctttggaaatccttcacgaccccaagatcaccgccatccaaccaaataagccgtctggtttcatcggatatagcttacattacgcccagttggcgtttcgcgtcctgttcttgaacgggccccagtccgatgcgcaggagcgaagagtccacccgaacgtcgccaacgctgtcaaggagctggaaatggctatcgaggagagcgccaaccccgacgcgatgttcttgttggccgagatgaacttctatggcaacttcacgcattcgcgcgacttcaagcaggcgtttcgatggtaccaggagcttgcttcgttgactggaaatagtacggcgcagtatatgatcggatttatgtatgcgacagggatcggcggtgcggttgaacgcgaccaagcgaaggccttgatgtatcacacttttgccgctgagggggggaatacaaggtcccagatgacgctcgcctatcgcttccactccggaattgggacaccgagaaactgcgacgaggcgaactactactacaaaatggttgcggataaggctattcggcactatcggtcaggtccgccgggtggcaataacatggatcgggaatcataccgctgggttgacagagagggtggggtgtacggagaaggagccagcatgtcgagttctgggccgaatgcgccacgagacatctcaaacactggcgcagaggctagcctagaggatatactggagtatctggacctcatgtcccggaagggcgaactgaaagctacaattagcctgggcaagatgcattacgagggggcccatggtctgcccaggaatttccgaagggcgatgaagtatttcaagactgtcacgaggcggtactggaacaaggatggctctgtcaatcctaaccacccatcgggggttgcgaaactagcgtcgaaagcagccggccatgtcgggacaatgtatcttcgtggtgaaggggtggagcagaattttggcactgccttaacatggttcaaacgtggactagccaatggcgacgcgctttgccaatatgaactcggcttaatgtatctgcatggatacggtgttcctaaagatgctttcagagctgcttcttacttcaaggccgcggctgagcaggatttcccagcggcagagacacggctaggcgcgctgttcctggatcagggcgatgttgaagcggctgcacgatatttcgagctggctgcgcgctggggatcgatggaggcgttttattatctggccgagctgtccaacggcggagttggtaggcgacgacactgtgggatggcaacagcctactataagatggttgcagagcgggctgaagctattcattcatctttcgccgaatcgaatgccgcctacgaaaatggcgataaagaacgagcagtcatcgctacaatgatggcagcggagcaaggatacgagaatgcgcagtccaacgtggcctatcttctggatgagcagaactccttgttctcactcgacgcgatcctgccttggggaggaaagtcccggcctagtctgcttcggaatgcggcgcaggctttgatctattggacccgttcagctaagcaggcgaatattgacgcgttgatcaaaatgggcgattactacctcgctggaataggagctgtagcggatgcggagaaggcatccacctgttatcataccgccgcggaagctcatcacagtgcgcaggcgtattggaatctcgggtggatgcatgagaacggtatcgcggtcgagcaagattttcacatggccaaaagatactatgacttggcactggaaaccaaccaagagtcgtatcttccggtgaaactgagcctgataaagctgcggatgcgaggctactggaaccgcatcaccaacgggaagatcaaccctatccaggaggaagagagtaagtcagatcgcggcatatcatgaagagacaactgacagcttgacagaccccaggccacaacgaagtttcaaggaatgggtcgccgcgttcatcgaaaacgacgaggaggaggaaaatctgcgagcacatctgtacaagcaagctaatggggaggacgacgatctcctctcgagcaatcgcctggagggcgaagacgagcgtgatgatgggtactacgacgatatggacctcgacatcgacgagagtctcctagaggctcttgttattctttctctagttgcgacgctgatgggacttctatacatgagacagcaacggaatcgacagcggcagaacgaggatgggggtgctggtgcgaatgctgcagccgatagaggagatcgcgggttgtttccaaggccgggagatccggattttgcaccatgggtagctggaggagtaggacattag

SEQ ID NO: 93 - DNA, 3819 bp, Unknown
  Newly identified micro-organism
atggccgactacgacgaagcgtacgaggaggagttctacgaggaggaggaggaaggaattacctcggaggactgctggacggtcatttcgtccttttttgacagcaaaggtctagtgtcgcagcagctggattccttcgatgagtttatctcgtcgacgatgcaagagttggtggaggaacagggtcaagtcgtggttgatcaaactctcccgcccgccgaagatgaagtcgatccggtggtgctccgtcgctacgaactcaagtttgggacagtcatgctctcaagaccttcagttacggaaggcgatggtgcgacgactatcatgttaccgcaggaggcccgtttgcggaatctcacctacgccagtccgctgtatctcgggatcacgaagagaataatggaaggtcgcgaacgaatggtggctgatggtgaggacggcgatgcgggtgatttagatgagcggagagcgaaaggtacatacctccagtgggagcagaagcagctttctgaagaccaagcgaaggaggaaactgttttcattggaaagatacccattatgctcaagtctaagtactgcattctcaaggacttgaacgagcaggcgctctacaattgggacgaatgcccctatgattctggtggctactttatcatcaacggaagcgagaaggtcctgatcgcgcaagagcgcagcgcagggaatatcgtccaggttttcaagaaggcgcctccgagtccgactccatatactgctgaaatccgaagtgccgtcgaaaagggttcgaggcttctctcgcagttatctcttaaactgtttgcgaagggagacagcgcaaaaggtggatttggtccgacgattagatcgacgctaccatatgtgaaaaccgacatccctatcgtggtcgtgttcagagctctcggagttgtgtccgacgaggatatcctcaaccacatctgctacgaccggaatgatacccctatgttggagatgctgaagccgtgtatcgaagagggcttcgtcattcaagaccgtgaagtcgctcttgatttcatcgctaagcgagggtctacacagtcaagtatgaatcacgagcggcgtgtcagatacgccagggaaatcatgcagaaggagttccttccgcatatttcgcagagcgagggaagcgagacccggaaggcgttcttcttgggatacatggtacacagactcttgcagtgcgccttgggtcgtcgggatgttgatgatcgtgatcattttggcaagaagcgcctcgatcttgccggtccgctactagcaaatctcttccgtgttttgttcacaagggttacgagggacctacagcggtatgtgcagcgatgcgtggagagtggtcgagagatctacttgaacattggtatcaaggctagcaccttgaccggaggcctgaaatacgcgcttgcaacaggaaactggggtgagcagaagaaggccgcaagctccaaagctggcgtgtcgcaggtcctgagtcgttacacttacgcatctacgctgtcacatcttcgtcggaccaacacccccatcggtcgcgacgggaagatcgcaaagccacggcagcttcataacacccactggggcttggtctgtccgtcagagacgccggaaggccaggcatgcggcctcgtcaagaacctggcgctcatgtgctatattactgtcggtacacccagcgaaccgattatcgacttcatgatccagcgcaacatggaggtactggaagagttcgagccgcaagtaacaccgaatgcgacaaaggtgtttgtaaacggtgtctgggttggtatccaccgcgacccgtctcaccttgtgagcaccatgctctctctgcgcaggcgcaacatgatttcccacgaggtcagtttgattcgggatatccgtgagcgagaattcaaaatcttcaccgacgctggtcgcgtatcgcggccgctgttcgtgatagacaatgacccgaagagcgagaattctggatctctcgtgctcagcaaggaacacatccgaaaactagagcaggataaggagctgcctccggatctggatccagaagagcgtagggagcgatacttcggatgggacggccttgtgaaatcgggcgtcgtggagtatgtcgatgcggaggaggaggaaacgatcatgatcgtgatgaccccggaggaccttgagatcgggaaacagcttcaggcaggatatagtctcccggaggagatcgatcctcataagcgtgtgagatcggttctcactcaaagagcacatacttggacgcactgcgagatccacccgagtatgattctgggtgtttgtgccagtatcattccgttcccggatcataaccagtcgcctcgtaacacttaccaagcagcaatgggcaaacaagccatgggcgtgttcttgaccaactttgaccagcgcatggagacgatgatgaatatcctttactatccccagaaacccctagcaacgacacgatcgatggagttcctccggttccgagagctgcctgccgggcagaatgccatcgtcgctattgcgtgctattctggatacaaccaggaggactcggttatcatgaaccaaagcagtatcgaccgcgggctcttccgaagcttgttctaccggacgtacaacgatgctgagaagatggttggattgacggtggttgagcgattcgagaggccgatgcggactgatacgattggcatgaggaaagggacatacgataagattgacgaggatggcatcattgccccaggcgtgcgcgtgtccggagaggacatcatcattggcaagacggcgcctttggcaccggaggcggaggagctcggccagagaaccaaagcccataccaaactggacgtgtcaacaccactgcgaagcacggagagtggtattgtggataaggttcttgtttcgaccggcagtgacgacctcaagtttgtcaaggtccgtatgaggacgactaagatcccccagattggtgataagttcgcttctcgccacgggcaaaagggtacgattggtgttacgtaccggcaggaagacatgccgtttactcgcgaaggcgtggtaccggacctcatcatcaaccctcatgctatcccatcgcgtatgacgattgcccacttgattgagtgtcagctcagcaaggtgtcggcgctgcgagggttcgaaggtgacgcgacgccgtttacggatgtcactgtagattcaatatcgcgcctgctccgcgagcacgggtatcagtcgcgtgggttcgaggtgatgtataacggacacacgggacgcaagctggttgcgcaggtcttcctgggaccgacgtactaccagcggctgcgacacatggtggatgacaagatccacgctcgtgcacgagggccgacacagatcctgacacgacagccggtggagggtagggcacgagatggtggactacgattcggtgagatggagcgcgactgtatgatcgcgcatggagccagcgcattcctgaaggagcggttatttgacgtatccgatccattccgagtccacatctgcgatgattgtgggctaatgacgccggttgcgtaagtcaacgatctgatacttcttatattgacagcacctgggactaactagagcagtaaactgaagaaaggactattcgagtgtcgactgtgcaacaacaagcaccggatctcgcaggtccatatcccatatgccgccaagcttctgttccaagaactggcctcgatgaatatcgcggcacgcatgtttaccgatcgttctggggtgtctgtacggtag

SEQ ID NO: 94 - DNA, 2589 bp, Unknown
  Newly identified micro-organism
atggctctccttcagtaccctgcgcccgttgactatacggcgcagctcaatgctttcaaggactttcttcagcacttcaagaccttcgagtcggcatccgaatcggcggcaacggaagctattgaggatctacatatcgatggcgatggcaccagcgatgaatatgattttatggatgacgtggaggatgagaacggggagcagagacctggtagaaggcatcgcgaaccgaagcacaagtacatgcagatgctacaagatgtcgcagatcgggaacggacaaatgttctcattgagctggatgaccttttaattgtaagcgatcagtactctagtgtctatcactactaactttcggacgcagttcgaaagatcactctctgaggagacaaatttgaaactggtcgagtctgtgcaaagaaataccaagcgctatattgatgtgttttctcaggcggtagacgccgtcatgcccaaagagactaaggaagtaacgtacgctttgcccagaggaatacaatggacgcgactaactcgcacaggttcaaagatgatgtcctcgatgttatcatgtcgcaacgcgagaagcgcaatgaagccatgaacttggccatgcagaccgatatggatgctgccgcaactccttcgattttccctcctgaattgacccgtcgatacaccctcaactttaagccggttacactctccgggtccagcagcgaacgtgattctaaggcgctcgcagtccggaatgttcgagctgaacatcttggcagtctcataaccgtccgtggcataacaacccgggtgtcagatgtcaagccggcagtccagataaacgcctatgcatgtgatcggtgtggctgtgaggtgttccagccgattaccacgaaacaattcctcccgctgacagagtgcttgtctgaggaatgtatgaagaacaactccaaggggcagctgttcctctccacccgtgcatcgaaatttgttccattccaagaggtgaagatccaggagatggcggaccaggtccctgttggccatatcccgcggacattgaccatccactgtcacggaagtctcacacggcaactcaatcctggggactatgttgatatcgcgggaattttccttcctattccctacaccggtttcagagctatccgcgctggtttgttgacggacacttacatggaagcccagcatatcactcagcataagaaagcatacaacgatctcgtgatggagagtcgtactcttcgaaagatcgaacagtaccaaagatcgggccagatgtatgaatacctgtcacggtccattgctcctgaaattttcggtcacatggatatcaagaaagccctactactgcttctaatcgggggagttacgaaggaaatgggcgacggcatgcacatccgtggagatatcaatatctgtctgatgggagatcctggtgtggcaaagtcccagctgctgaaatatatcgctaaggtcgctcctcgaggcgtatacacaaccggccgagggagtagcggtgtcggtctcacagcagcagtcatgagagaccctgtgaccgacgagatggttctggagggaggagcgctggttctagcagacaatggcatttgctgtattgacgagttcgacaaaatggaagacggggataggacggccatccacgaggtgatggagcagcagaccatttcgatttcgaaggcagggattacaacgaccctgaacgcacgtacatccatcctggcggccgcaaacccgttgtatgggcgatacaacccacgagtgtctcccgtggaaaacatcaaccttcctgcggctctactctctcgtttcgacgtcaccttccttgttcttgataccccgtcacgggatgcggacgaaaacctggcgagtcacgtcacgtacgttcatatgcacaataagcaccccgagaacgaagacacgccggccgtcttctctccccacgaagtccgtcaatacatcgccaaggcgcggacgtatcggccggtcgtgccgtccgcgatctctgactacatggttggagcatacgtgcagatgcggaagcaacagaagaaggatgagggtagcaagagacagttttcaccagtcactccacgtacactgctcggtgtgatccgtctgtcgcaggcgcttgcgcgcttaagattcagtgaccaggtggtcatggaggacgtggacgaggcgctacgtctcattgcggttagcaaggcgtcgctcgagagcgaggaccagagcggcgttgatcacaccccgagcagcaagatctatagtttgatccggaacatgcgagaaagtggtgcagcggccgtgggcgacggtgaagacggggagctgagcatgagaagggtcagggagagagtgttggccaagggattcacggaagaccagctgactatggcgatcgacgaatacgccaacttggatgtaagttgttgctcggtatatgaagtctgcatttccactgacgatcaatcacaggtctggcaggtcacggctggagggacgcgacttgtatttatcgaggcggatggagttgagaggatggagatgtga